European Patent Application EP 4 464 715 A2, published November 20, 2024. Title: BICYCLIC PEPTIDE LIGANDS SPECIFIC FOR NECTIN-4. Applicant: BicycleTx Limited. The sequence listing filed with the application follows.

SEQUENCE LISTING (217 sequences)

SEQ ID NO: 1 - protein, 15 aa, synthetic construct
  REGION 1..15: note = synthetic
CPFGCMKNWSWPIWC

SEQ ID NO: 2 - protein, 15 aa, synthetic construct
  REGION 1..15: note = synthetic
CPFGCMRNWSWPIWC

SEQ ID NO: 3 - protein, 15 aa, synthetic construct
  REGION 1..15: note = synthetic
  SITE 6: note = Xaa - neopentyl glycine
CPFGCXKNWSWPIWC

SEQ ID NO: 4 - protein, 15 aa, synthetic construct
  REGION 1..15: note = synthetic
  SITE 6: note = Xaa - homoleucine
CPFGCXKNWSWPIWC

SEQ ID NO: 5 - protein, 15 aa, synthetic construct
  REGION 1..15: note = synthetic
CPFGCIKNWSWPIWC

SEQ ID NO: 6 - protein, 15 aa, synthetic construct
  REGION 1..15: note = synthetic
CPFACMKNWSWPIWC

SEQ ID NO: 7 - protein, 15 aa, synthetic construct
  REGION 1..15: note = synthetic
CPFGCQKNWSWPIWC

SEQ ID NO: 8 - protein, 15 aa, synthetic construct
  REGION 1..15: note = synthetic
CPFGCMKNWSDPIWC

SEQ ID NO: 9 - protein, 15 aa, synthetic construct
  REGION 1..15: note = synthetic
  SITE 14: note = Xaa - 1-naphthyl alanine
CPFGCMKNWSWPIXC

SEQ ID NO: 10 - protein, 15 aa, synthetic construct
  REGION 1..15: note = synthetic
  SITE 2: note = Xaa - hydroxyproline
CXFGCMKNWSWPIWC

SEQ ID NO: 11 - protein, 15 aa, synthetic construct
  REGION 1..15: note = synthetic
CPYGCMKNWSWPIWC

SEQ ID NO: 12 - protein, 15 aa, synthetic construct
  REGION 1..15: note = synthetic
CPFGCMSNWSWPIWC

SEQ ID NO: 13 - protein, 15 aa, synthetic construct
  REGION 1..15: note = synthetic
CPFGCMDNWSWPIWC

SEQ ID NO: 14 - protein, 15 aa, synthetic construct
  REGION 1..15: note = synthetic
  SITE 7: note = Xaa - homoarginine
CPFGCMXNWSWPIWC

SEQ ID NO: 15 - protein, 15 aa, synthetic construct
  REGION 1..15: note = synthetic
CPFGCMKDWSWPIWC

SEQ ID NO: 16 - protein, 15 aa, synthetic construct
  REGION 1..15: note = synthetic
CPFGCMKHWSWPIWC

SEQ ID NO: 17 - protein, 15 aa, synthetic construct
  REGION 1..15: note = synthetic
  SITE 9: note = Xaa - 1-naphthyl alanine
CPFGCMKNXSWPIWC

SEQ ID NO: 18 - protein, 15 aa, synthetic construct
  REGION 1..15: note = synthetic
  SITE 9: note = Xaa - 2-naphthyl alanine
CPFGCMKNXSWPIWC

SEQ ID NO: 19 - protein, 15 aa, synthetic construct
  REGION 1..15: note = synthetic
CPFGCMKNWSTPIWC

SEQ ID NO: 20 - protein, 15 aa, synthetic construct
  REGION 1..15: note = synthetic
CPFGCMKNWSWPDWC

SEQ ID NO: 21 - protein, 15 aa, synthetic construct
  REGION 1..15: note = synthetic
  SITE 14: note = Xaa - 2-naphthyl alanine
CPFGCMKNWSWPIXC

SEQ ID NO: 22 - protein, 15 aa, synthetic construct
  REGION 1..15: note = synthetic
  SITE 7: note = Xaa - homoarginine
CPFGCMXNWSWPIWC

SEQ ID NO: 23 - protein, 15 aa, synthetic construct
  REGION 1..15: note = synthetic
  SITE 7: note = Xaa - N-acetyllysine
CPFGCMXNWSWPIWC

SEQ ID NO: 24 - protein, 15 aa, synthetic construct
  REGION 1..15: note = synthetic
CPFGCMKNWSAPIWC

SEQ ID NO: 25 - protein, 15 aa, synthetic construct
  REGION 1..15: note = synthetic
CPFGCMKNWSWPAWC

SEQ ID NO: 26 - protein, 15 aa, synthetic construct
  REGION 1..15: note = synthetic
CAFGCMKNWSWPIWC

SEQ ID NO: 27 - protein, 15 aa, synthetic construct
  REGION 1..15: note = synthetic
CPFGCMANWSWPIWC

SEQ ID NO: 28 - protein, 15 aa, synthetic construct
  REGION 1..15: note = synthetic
CPFGCMKAWSWPIWC

SEQ ID NO: 29 - protein, 15 aa, synthetic construct
  REGION 1..15: note = synthetic
  SITE 6: note = Xaa - Nle
CPFGCXKNWSWPIWC

SEQ ID NO: 30 - protein, 15 aa, synthetic construct
  REGION 1..15: note = synthetic
CPFGCMKNWAWPIWC

SEQ ID NO: 31 - protein, 13 aa, synthetic construct
  REGION 1..13: note = synthetic
CWPLDSYWCARIC

SEQ ID NO: 32 - protein, 13 aa, synthetic construct
  REGION 1..13: note = synthetic
CAPLDDYWCGRIC

SEQ ID NO: 33 - protein, 13 aa, synthetic construct
  REGION 1..13: note = synthetic
CAPLDDYWCDRIC

SEQ ID NO: 34 - protein, 13 aa, synthetic construct
  REGION 1..13: note = synthetic
CAPLSDYWCNRIC

SEQ ID NO: 35 - protein, 15 aa, synthetic construct
  REGION 1..15: note = synthetic
CVTTSYDCFLHLLGC

SEQ ID NO: 36 - protein, 15 aa, synthetic construct
  REGION 1..15: note = synthetic
CVTTSYDCWVRLGQC

SEQ ID NO: 37 - protein, 15 aa, synthetic construct
  REGION 1..15: note = synthetic
CVTTSYDCWVTLGHC

SEQ ID NO: 38 - protein, 15 aa, synthetic construct
  REGION 1..15: note = synthetic
  SITE 2: note = Xaa - P/A/hydroxyproline
  SITE 3: note = Xaa - F/Y
  SITE 4: note = Xaa - G/A
  REGION 6..8: note = Xaa - any amino acid
  SITE 9: note = Xaa - W/1-naphthyl alanine/2-naphthyl alanine
  SITE 10: note = Xaa - S/A
  SITE 11: note = Xaa - any amino acid
  SITE 13: note = Xaa - I/D/A
  SITE 14: note = Xaa - W/1-naphthyl alanine/2-naphthyl alanine
CXXXCXXXXXXPXXC

SEQ ID NO: 39 - protein, 13 aa, synthetic construct
  REGION 1..13: note = synthetic
  SITE 2: note = Xaa - W/A
  SITE 5: note = Xaa - D/S
  SITE 6: note = Xaa - S/D
  SITE 10: note = Xaa - any amino acid
CXPLXXYWCXRIC

SEQ ID NO: 40 - protein, 15 aa, synthetic construct
  REGION 1..15: note = synthetic
  SITE 9: note = Xaa - F/W
  SITE 10: note = Xaa - L/V
  SITE 11: note = Xaa - H/R/T
  SITE 13: note = Xaa - L/G
  SITE 14: note = Xaa - G/Q/H
CVTTSYDCXXXLXXC

SEQ ID NO: 41 - skipped

SEQ ID NO: 42 - protein, 13 aa, synthetic construct
  REGION 1..13: note = synthetic
  SITE 2: note = Xaa - W/A/Y
  SITE 3: note = Xaa - P/A
  SITE 5: note = Xaa - D/S/A
  SITE 6: note = Xaa - S/D/P/A
  SITE 8: note = Xaa - W/1-naphthyl alanine
  SITE 10: note = Xaa - any amino acid
  SITE 11: note = Xaa - R/homoarginine/A
CXXLXXYXCXXIC

SEQ ID NO: 43 - protein, 13 aa, synthetic construct
  REGION 1..13: note = synthetic
CWPLDPYWCGRIC

SEQ ID NO: 44 - protein, 13 aa, synthetic construct
  REGION 1..13: note = synthetic
CYPLSPYWCERIC

SEQ ID NO: 45 - protein, 15 aa, synthetic construct
  REGION 1..15: note = synthetic
CPFGCMETWSWPIWC

SEQ ID NO: 46 - protein, 15 aa, synthetic construct
  REGION 1..15: note = synthetic
CPFGCMRGWSWPIWC

SEQ ID NO: 47 - protein, 15 aa, synthetic construct
  REGION 1..15: note = synthetic
CPFGCMSGWSWPIWC

SEQ ID NO: 48 - protein, 15 aa, synthetic construct
  REGION 1..15: note = synthetic
CPFGCMEGWSWPIWC

SEQ ID NO: 49 - protein, 15 aa, synthetic construct
  REGION 1..15: note = synthetic
CPFGCMEDWSWPIWC

SEQ ID NO: 50 - protein, 15 aa, synthetic construct
  REGION 1..15: note = synthetic
CPFGCMPGWSWPIWC

SEQ ID NO: 51 - protein, 15 aa, synthetic construct
  REGION 1..15: note = synthetic
CPFGCMKSWSWPIWC

SEQ ID NO: 52 - protein, 15 aa, synthetic construct
  REGION 1..15: note = synthetic
CPFGCMKTWSWPIWC

SEQ ID NO: 53 - protein, 15 aa, synthetic construct
  REGION 1..15: note = synthetic
CPFGCMKGWSWPIWC

SEQ ID NO: 54 - protein, 15 aa, synthetic construct
  REGION 1..15: note = synthetic
CPFGCQEHWSWPIWC

SEQ ID NO: 55 - protein, 15 aa, synthetic construct
  REGION 1..15: note = synthetic
CPFGCIKSWSWPIWC

SEQ ID NO: 56 - protein, 15 aa, synthetic construct
  REGION 1..15: note = synthetic
CPFGCQEDWSWPIWC

SEQ ID NO: 57 - protein, 15 aa, synthetic construct
  REGION 1..15: note = synthetic
CPFGCMSDWSWPIWC

SEQ ID NO: 58 - protein, 13 aa, synthetic construct
  REGION 1..13: note = synthetic
CWPLDDYWCPRIC

SEQ ID NO: 59 - protein, 15 aa, synthetic construct
  REGION 1..15: note = synthetic
  SITE 7: note = Xaa - homoarginine
CPFGCMXNWSWPIWC

SEQ ID NO: 60 - protein, 15 aa, synthetic construct
  REGION 1..15: note = synthetic
  SITE 7: note = Xaa - N-acetyllysine
CPFGCMXNWSWPIWC

SEQ ID NO: 61 - protein, 15 aa, synthetic construct
  REGION 1..15: note = synthetic
  SITE 7: note = Xaa - N-acetyllysine
CPFGCMXSWSWPIWC

SEQ ID NO: 62 - protein, 15 aa, synthetic construct
  REGION 1..15: note = synthetic
  SITE 6: note = Xaa - Nle
CPFGCXKSWSWPIWC

SEQ ID NO: 63 - protein, 15 aa, synthetic construct
  REGION 1..15: note = synthetic
  SITE 7: note = Xaa - homoarginine
CPFGCMXSWSWPIWC

SEQ ID NO: 64 - protein, 15 aa, synthetic construct
  REGION 1..15: note = synthetic
  SITE 7: note = Xaa - D-lysine
CPFGCMXSWSWPIWC

SEQ ID NO: 65 - protein, 13 aa, synthetic construct
  REGION 1..13: note = synthetic
  SITE 11: note = Xaa - homoarginine
CAPLSDYWCNXIC

SEQ ID NO: 66 - protein, 15 aa, synthetic construct
  REGION 1..15: note = synthetic
  SITE 3: note = Xaa - D-alanine
CPXGCMKNWSWPIWC

SEQ ID NO: 67 - protein, 15 aa, synthetic construct
  REGION 1..15: note = synthetic
  SITE 4: note = Xaa - D-alanine
CPFXCMKNWSWPIWC

SEQ ID NO: 68 - protein, 15 aa, synthetic construct
  REGION 1..15: note = synthetic
  SITE 7: note = Xaa - D-alanine
CPFGCMXNWSWPIWC

SEQ ID NO: 69 - protein, 15 aa, synthetic construct
  REGION 1..15: note = synthetic
  SITE 8: note = Xaa - D-alanine
CPFGCMKXWSWPIWC

SEQ ID NO: 70 - protein, 15 aa, synthetic construct
  REGION 1..15: note = synthetic
  SITE 9: note = Xaa - D-alanine
CPFGCMKNXSWPIWC

SEQ ID NO: 71 - protein, 15 aa, synthetic construct
  REGION 1..15: note = synthetic
  SITE 13: note = Xaa - D-alanine
CPFGCMKNWSWPXWC

SEQ ID NO: 72 - protein, 15 aa, synthetic construct
  REGION 1..15: note = synthetic
  SITE 2: note = Xaa - D-alanine
CXFGCMKNWSWPIWC

SEQ ID NO: 73 - protein, 15 aa, synthetic construct
  REGION 1..15: note = synthetic
  SITE 6: note = Xaa - t-butyl-alanine
CPFGCXKNWSWPIWC

SEQ ID NO: 74 - protein, 15 aa, synthetic construct
  REGION 1..15: note = synthetic
  SITE 6: note = Xaa - homoleucine
CPFGCXKNWSWPIWC

SEQ ID NO: 75 - protein, 15 aa, synthetic construct
  REGION 1..15: note = synthetic
  SITE 14: note = Xaa - 1-naphthyl alanine
CPFGCMKNWSWPIXC

SEQ ID NO: 76 - protein, 15 aa, synthetic construct
  REGION 1..15: note = synthetic
  SITE 4: note = Xaa - D-Aspartic acid
  SITE 7: note = Xaa - homoarginine
CPFXCMXNWSWPIWC

SEQ ID NO: 77 - protein, 15 aa, synthetic construct
  REGION 1..15: note = synthetic
  SITE 4: note = Xaa - D-alanine
  SITE 7: note = Xaa - homoarginine
CPFXCMXNWSWPIWC

SEQ ID NO: 78 - protein, 15 aa, synthetic construct
  REGION 1..15: note = synthetic
  SITE 3: note = Xaa - 3-methyl-phenylalanine
CPXGCMKNWSWPIWC

SEQ ID NO: 79 - protein, 15 aa, synthetic construct
  REGION 1..15: note = synthetic
  SITE 3: note = Xaa - 4-methyl-phenylalanine
CPXGCMKNWSWPIWC

SEQ ID NO: 80 - protein, 15 aa, synthetic construct
  REGION 1..15: note = synthetic
  SITE 3: note = Xaa - homophenylalanine
CPXGCMKNWSWPIWC

SEQ ID NO: 81 - protein, 15 aa, synthetic construct
  REGION 1..15: note = synthetic
  SITE 4: note = Xaa - D-Aspartic acid
CPFXCMKNWSWPIWC

SEQ ID NO: 82 - protein, 15 aa, synthetic construct
  REGION 1..15: note = synthetic
  SITE 6: note = Xaa - homoserine-methyl
CPFGCXKNWSWPIWC

SEQ ID NO: 83 - protein, 15 aa, synthetic construct
  REGION 1..15: note = synthetic
  SITE 9: note = Xaa - azatryptophan
CPFGCMKNXSWPIWC

SEQ ID NO: 84 - protein, 15 aa, synthetic construct
  REGION 1..15: note = synthetic
CPFGCMKNWSFPIWC

SEQ ID NO: 85 - protein, 15 aa, synthetic construct
  REGION 1..15: note = synthetic
CPFGCMKNWSYPIWC

SEQ ID NO: 86 - protein, 15 aa, synthetic construct
  REGION 1..15: note = synthetic
  SITE 11: note = Xaa - 1-naphthyl alanine
CPFGCMKNWSXPIWC

SEQ ID NO: 87 - protein, 15 aa, synthetic construct
  REGION 1..15: note = synthetic
  SITE 11: note = Xaa - 2-naphthyl alanine
CPFGCMKNWSXPIWC

SEQ ID NO: 88 - protein, 15 aa, synthetic construct
  REGION 1..15: note = synthetic
  SITE 11: note = Xaa - azatryptophan
CPFGCMKNWSXPIWC

SEQ ID NO: 89 - protein, 15 aa, synthetic construct
  REGION 1..15: note = synthetic
  SITE 12: note = Xaa - azetidine
CPFGCMKNWSWXIWC

SEQ ID NO: 90 - protein, 15 aa, synthetic construct
  REGION 1..15: note = synthetic
  SITE 12: note = Xaa - pipecolic acid
CPFGCMKNWSWXIWC

SEQ ID NO: 91 - protein, 15 aa, synthetic construct
  REGION 1..15: note = synthetic
CPFGCMKNWSWPIFC

SEQ ID NO: 92 - protein, 15 aa, synthetic construct
  REGION 1..15: note = synthetic
CPFGCMKNWSWPIYC

SEQ ID NO: 93 - protein, 15 aa, synthetic construct
  REGION 1..15: note = synthetic
  SITE 14: note = Xaa - azatryptophan
CPFGCMKNWSWPIXC

SEQ ID NO: 94 - protein, 15 aa, synthetic construct
  REGION 1..15: note = synthetic
CGFGCMKNWSWPIWC

SEQ ID NO: 95 - protein, 15 aa, synthetic construct
  REGION 1..15: note = synthetic
  SITE 2: note = Xaa - azetidine
CXFGCMKNWSWPIWC

SEQ ID NO: 96 - protein, 15 aa, synthetic construct
  REGION 1..15: note = synthetic
  SITE 4: note = Xaa - N-acetyllysine
CPFXCMKNWSWPIWC

SEQ ID NO: 97 - protein, 15 aa, synthetic construct
  REGION 1..15: note = synthetic
CPFGCLKNWSWPIWC

SEQ ID NO: 98 - protein, 15 aa, synthetic construct
  REGION 1..15: note = synthetic
  SITE 6: note = Xaa - MetO2
CPFGCXKNWSWPIWC

SEQ ID NO: 99 - protein, 15 aa, synthetic construct
  REGION 1..15: note = synthetic
CPFGCMPNWSWPIWC

SEQ ID NO: 100 - protein, 15 aa, synthetic construct
  REGION 1..15: note = synthetic
CPFGCMQNWSWPIWC

SEQ ID NO: 101 - protein, 15 aa, synthetic construct
  REGION 1..15: note = synthetic
CPFGCMKNWSWPPWC

SEQ ID NO: 102 - protein, 15 aa, synthetic construct
  REGION 1..15: note = synthetic
  SITE 3: note = Xaa - 2-pyridylalanine
CPXGCMKNWSWPIWC

SEQ ID NO: 103 - protein, 13 aa, synthetic construct
  REGION 1..13: note = synthetic
CAALSDYWCNRIC

SEQ ID NO: 104 - protein, 13 aa, synthetic construct
  REGION 1..13: note = synthetic
CAPLADYWCNRIC

SEQ ID NO: 105 - protein, 13 aa, synthetic construct
  REGION 1..13: note = synthetic
CAPLSAYWCNRIC

SEQ ID NO: 106 - protein, 13 aa, synthetic construct
  REGION 1..13: note = synthetic
CAPLSDYWCARIC

SEQ ID NO: 107 - protein, 13 aa, synthetic construct
  REGION 1..13: note = synthetic
CAPLSDYWCNAIC

SEQ ID NO: 108 - protein, 13 aa, synthetic construct
  REGION 1..13: note = synthetic
  SITE 5: note = Xaa - D-alanine
CAPLXDYWCNRIC

SEQ ID NO: 109 - protein, 13 aa, synthetic construct
  REGION 1..13: note = synthetic
  SITE 6: note = Xaa - D-alanine
CAPLSXYWCNRIC

SEQ ID NO: 110 - protein, 13 aa, synthetic construct
  REGION 1..13: note = synthetic
  SITE 10: note = Xaa - D-alanine
CAPLSDYWCXRIC

SEQ ID NO: 111 - protein, 15 aa, synthetic construct
  REGION 1..15: note = synthetic
  SITE 9: note = Xaa - 1-naphthyl alanine
CPFGCMKNXSWPIWC

SEQ ID NO: 112 - protein, 15 aa, synthetic construct
  REGION 1..15: note = synthetic
  SITE 9: note = Xaa - 2-naphthyl alanine
CPFGCMKNXSWPIWC

SEQ ID NO: 113 - protein, 15 aa, synthetic construct
  REGION 1..15: note = synthetic
  SITE 14: note = Xaa - 2-naphthyl alanine
CPFGCMKNWSWPIXC

SEQ ID NO: 114 - protein, 15 aa, synthetic construct
  REGION 1..15: note = synthetic
  SITE 2: note = Xaa - hydroxyproline
CXFGCMKNWSWPIWC

SEQ ID NO: 115 - protein, 15 aa, synthetic construct
  REGION 1..15: note = synthetic
  SITE 4: note = Xaa - D-Aspartic acid
  SITE 7: note = Xaa - homoarginine
CPFXCMXNWSTPIWC

SEQ ID NO: 116 - protein, 15 aa, synthetic construct
  REGION 1..15: note = synthetic
  SITE 4: note = Xaa - D-Aspartic acid
  SITE 7: note = Xaa - homoarginine
  SITE 8: note = Xaa - D-lysine
CPFXCMXXWSTPIWC

SEQ ID NO: 117 - protein, 15 aa, synthetic construct
  REGION 1..15: note = synthetic
  SITE 4: note = Xaa - D-Aspartic acid
  SITE 7: note = Xaa - homoarginine
CPFXCMXNWSTPKWC

SEQ ID NO: 118 - protein, 15 aa, synthetic construct
  REGION 1..15: note = synthetic
  SITE 2: note = Xaa - 4-amino-proline
  SITE 4: note = Xaa - D-Aspartic acid
  SITE 7: note = Xaa - homoarginine
CXFXCMXNWSTPIWC

SEQ ID NO: 119 - protein, 15 aa, synthetic construct
  REGION 1..15: note = synthetic
  SITE 4: note = Xaa - D-Aspartic acid
CPFXCMKNWSTPIWC

SEQ ID NO: 120 - protein, 15 aa, synthetic construct
  REGION 1..15: note = synthetic
  SITE 4: note = Xaa - D-lysine
  SITE 7: note = Xaa - homoarginine
CPFXCMXNWSTPIWC

SEQ ID NO: 121 - protein, 15 aa, synthetic construct
  REGION 1..15: note = synthetic
  SITE 4: note = Xaa - D-Aspartic acid
  SITE 7: note = Xaa - homoarginine
CPFXCKXNWSTPIWC

SEQ ID NO: 122 - protein, 15 aa, synthetic construct
  REGION 1..15: note = synthetic
  SITE 4: note = Xaa - D-Aspartic acid
  SITE 7: note = Xaa - homoarginine
CPFXCMXKWSTPIWC

SEQ ID NO: 123 - protein, 15 aa, synthetic construct
  REGION 1..15: note = synthetic
  SITE 2: note = Xaa - oxazolidine-4-carboxylic acid
  SITE 4: note = Xaa - D-Aspartic acid
  SITE 7: note = Xaa - homoarginine
CXFXCMXNWSTPIWC

SEQ ID NO: 124 - protein, 15 aa, synthetic construct
  REGION 1..15: note = synthetic
  SITE 4: note = Xaa - D-Aspartic acid
  SITE 7: note = Xaa - homoarginine
  SITE 8: note = Xaa - Thienyl-alanine
CPFXCMXXWSTPIWC

SEQ ID NO: 125 - protein, 15 aa, synthetic construct
  REGION 1..15: note = synthetic
  SITE 4: note = Xaa - D-Aspartic acid
  SITE 7: note = Xaa - homoarginine
  SITE 8: note = Xaa - Beta-(4-thiazolyl)-alanine
CPFXCMXXWSTPIWC

SEQ ID NO: 126 - protein, 15 aa, synthetic construct
  REGION 1..15: note = synthetic
  SITE 4: note = Xaa - D-Aspartic acid
  SITE 7: note = Xaa - homoarginine
  SITE 8: note = Xaa - 3-(1,2,4-Triazol-1-yl)-alanine
CPFXCMXXWSTPIWC

SEQ ID NO: 127 - protein, 15 aa, synthetic construct
  REGION 1..15: note = synthetic
  SITE 4: note = Xaa - D-Aspartic acid
  SITE 7: note = Xaa - homoarginine
  SITE 11: note = Xaa - 3-(1,2,4-Triazol-1-yl)-alanine
CPFXCMXNWSXPIWC

SEQ ID NO: 128 - protein, 15 aa, synthetic construct
  REGION 1..15: note = synthetic
  SITE 4: note = Xaa - D-Aspartic acid
  SITE 7: note = Xaa - homoarginine
  SITE 12: note = Xaa - oxazolidine-4-carboxylic acid
CPFXCMXNWSTXIWC

SEQ ID NO: 129 - protein, 15 aa, synthetic construct
  REGION 1..15: note = synthetic
  SITE 3: note = Xaa - 3,4-dihydroxy-phenylalanine
  SITE 4: note = Xaa - D-Aspartic acid
  SITE 7: note = Xaa - homoarginine
CPXXCMXNWSTPIWC

SEQ ID NO: 130 - protein, 15 aa, synthetic construct
  REGION 1..15: note = synthetic
  SITE 4: note = Xaa - D-Aspartic acid
  SITE 7: note = Xaa - homoarginine
  SITE 11: note = Xaa - 3,4-dihydroxy-phenylalanine
CPFXCMXNWSXPIWC

SEQ ID NO: 131 - protein, 15 aa, synthetic construct
  REGION 1..15: note = synthetic
  SITE 4: note = Xaa - D-Aspartic acid
  SITE 7: note = Xaa - homoarginine
  SITE 11: note = Xaa - dioxo-4-tetrahydrothiopyranylacetic acid
CPFXCMXNWSXPIWC

SEQ ID NO: 132 - protein, 15 aa, synthetic construct
  REGION 1..15: note = synthetic
  SITE 4: note = Xaa - D-Aspartic acid
  SITE 7: note = Xaa - homoarginine
  SITE 13: note = Xaa - dioxo-4-tetrahydrothiopyranylacetic acid
CPFXCMXNWSTPXWC

SEQ ID NO: 133 - protein, 15 aa, synthetic construct
  REGION 1..15: note = synthetic
  SITE 4: note = Xaa - D-Aspartic acid
  SITE 7: note = Xaa - homoarginine
  SITE 9: note = Xaa - 5-fluoro-L-tryptophan acid
CPFXCMXNXSTPIWC

SEQ ID NO: 134 - protein, 15 aa, synthetic construct
  REGION 1..15: note = synthetic
  SITE 4: note = Xaa - D-Aspartic acid
  SITE 7: note = Xaa - homoarginine
  SITE 14: note = Xaa - 5-fluoro-L-tryptophan acid
CPFXCMXNWSTPIXC

SEQ ID NO: 135 - protein, 15 aa, synthetic construct
  REGION 1..15: note = synthetic
  SITE 4: note = Xaa - D-Aspartic acid
  SITE 7: note = Xaa - homoarginine
  SITE 11: note = Xaa - tetrahydropyran-4-propanoic acid
CPFXCMXNWSXPIWC

SEQ ID NO: 136 - protein, 15 aa, synthetic construct
  REGION 1..15: note = synthetic
  SITE 4: note = Xaa - D-Aspartic acid
  SITE 7: note = Xaa - homoarginine
  SITE 13: note = Xaa - tetrahydropyran-4-propanoic acid
CPFXCMXNWSTPXWC

SEQ ID NO: 137 - protein, 15 aa, synthetic construct
  REGION 1..15: note = synthetic
  SITE 2: note = Xaa - 4,4-difluoroproline
  SITE 4: note = Xaa - D-Aspartic acid
  SITE 7: note = Xaa - homoarginine
CXFXCMXNWSTPIWC

SEQ ID NO: 138 - protein, 15 aa, synthetic construct
  REGION 1..15: note = synthetic
  SITE 2: note = Xaa - octahydroindolecarboxylic acid
  SITE 4: note = Xaa - D-Aspartic acid
  SITE 7: note = Xaa - homoarginine
CXFXCMXNWSTPIWC

SEQ ID NO: 139 - protein, 15 aa, synthetic construct
  REGION 1..15: note = synthetic
  SITE 4: note = Xaa - D-phenylalanine
  SITE 7: note = Xaa - homoarginine
CPFXCMXNWSTPIWC

SEQ ID NO: 140 - protein, 15 aa, synthetic construct
  REGION 1..15: note = synthetic
  SITE 4: note = Xaa - D-glutamic acid
  SITE 7: note = Xaa - homoarginine
CPFXCMXNWSTPIWC

SEQ ID NO: 141 - protein, 15 aa, synthetic construct
  REGION 1..15: note = synthetic
  SITE 4: note = Xaa - D-glutamine
  SITE 7: note = Xaa - homoarginine
CPFXCMXNWSTPIWC

SEQ ID NO: 142 - protein, 15 aa, synthetic construct
  REGION 1..15: note = synthetic
  SITE 4: note = Xaa - D-leucine
  SITE 7: note = Xaa - homoarginine
CPFXCMXNWSTPIWC

SEQ ID NO: 143 - protein, 15 aa, synthetic construct
  REGION 1..15: note = synthetic
  SITE 4: note = Xaa - D-serine
  SITE 7: note = Xaa - homoarginine
CPFXCMXNWSTPIWC

SEQ ID NO: 144 - protein, 15 aa, synthetic construct
  REGION 1..15: note = synthetic
  SITE 4: note = Xaa - D-Aspartic acid
  SITE 7: note = Xaa - homoarginine
  SITE 10: note = Xaa - homoserine
CPFXCMXNWXTPIWC

SEQ ID NO: 145 - protein, 15 aa, synthetic construct
  REGION 1..15: note = synthetic
  SITE 4: note = Xaa - D-Aspartic acid
  SITE 7: note = Xaa - homoarginine
  SITE 13: note = Xaa - cyclopentyl-glycine
CPFXCMXNWSTPXWC

SEQ ID NO: 146 - protein, 15 aa, synthetic construct
  REGION 1..15: note = synthetic
  SITE 4: note = Xaa - D-Aspartic acid
  SITE 7: note = Xaa - homoarginine
  SITE 13: note = Xaa - cyclopropyl-alanine
CPFXCMXNWSTPXWC

SEQ ID NO: 147 - protein, 15 aa, synthetic construct
  REGION 1..15: note = synthetic
  SITE 4: note = Xaa - D-Aspartic acid
  SITE 7: note = Xaa - homoarginine
  SITE 13: note = Xaa - 3-cyclohexyl-alanine
CPFXCMXNWSTPXWC

SEQ ID NO: 148 - protein, 15 aa, synthetic construct
  REGION 1..15: note = synthetic
  SITE 4: note = Xaa - D-Aspartic acid
  SITE 6: note = Xaa - homoglutamine
  SITE 7: note = Xaa - homoarginine
CPFXCXXNWSTPIWC

SEQ ID NO: 149 - protein, 15 aa, synthetic construct
  REGION 1..15: note = synthetic
  SITE 4: note = Xaa - D-Aspartic acid
  SITE 6: note = Xaa - cyclopentyl-glycine
  SITE 7: note = Xaa - homoarginine
CPFXCXXNWSTPIWC

SEQ ID NO: 150 - protein, 15 aa, synthetic construct
  REGION 1..15: note = synthetic
  SITE 4: note = Xaa - D-Aspartic acid
  SITE 7: note = Xaa - homoarginine
  SITE 9: note = Xaa - Methyl Tryptophan
CPFXCMXNXSTPIWC

SEQ ID NO: 151 - protein, 15 aa, synthetic construct
  REGION 1..15: note = synthetic
  SITE 4: note = Xaa - D-Aspartic acid
  SITE 5: note = Xaa - N-methyl-Cysteine
  SITE 7: note = Xaa - homoarginine
CPFXXMXNWSTPIWC

SEQ ID NO: 152 - protein, 14 aa, synthetic construct
  REGION 1..14: note = synthetic
  SITE 4: note = Xaa - D-Aspartic acid
  SITE 6: note = Xaa - homoarginine
  SITE 10: note = Xaa - N-methyl-Threonine
CPFXCXNWSXPIWC

SEQ ID NO: 153 - protein, 13 aa, synthetic construct
  REGION 1..13: note = synthetic
  SITE 8: note = Xaa - 1-naphthyl alanine
CAPLSDYXCNRIC

SEQ ID NO: 154 - protein, 13 aa, synthetic construct
  REGION 1..13: note = synthetic
  SITE 10: note = Xaa - D-Aspartic acid
CAPLSDYWCXRIC

SEQ ID NO: 155 - protein, 15 aa, synthetic construct
  REGION 1..15: note = synthetic
  SITE 3: note = Xaa - 1-naphthyl alanine
  SITE 4: note = Xaa - D-Aspartic acid
  SITE 7: note = Xaa - homoarginine
CPXXCMXNWSTPIWC

SEQ ID NO: 156 - protein, 15 aa, synthetic construct
  REGION 1..15: note = synthetic
  SITE 3: note = Xaa - 2-naphthyl alanine
  SITE 4: note = Xaa - D-Aspartic acid
  SITE 7: note = Xaa - homoarginine
CPXXCMXNWSTPIWC

SEQ ID NO: 157 - protein, 15 aa, synthetic construct
  REGION 1..15: note = synthetic
  SITE 3: note = Xaa - 4,4-biphenylalanine
  SITE 4: note = Xaa - D-Aspartic acid
  SITE 7: note = Xaa - homoarginine
CPXXCMXNWSTPIWC

SEQ ID NO: 158 - protein, 15 aa, synthetic construct
  REGION 1..15: note = synthetic
  SITE 4: note = Xaa - D-Aspartic acid
  SITE 7: note = Xaa - homoarginine
CPFXCMXNWSTPPWC

SEQ ID NO: 159 - protein, 15 aa, synthetic construct
  REGION 1..15: note = synthetic
  SITE 4: note = Xaa - D-Aspartic acid
  SITE 7: note = Xaa - homoarginine
  SITE 13: note = Xaa - hydroxyproline
CPFXCMXNWSTPXWC

SEQ ID NO: 160 - protein, 15 aa, synthetic construct
  REGION 1..15: note = synthetic
  SITE 4: note = Xaa - D-Aspartic acid
  SITE 7: note = Xaa - homoarginine
CPFXCLXNWSTPPWC

SEQ ID NO: 161 - protein, 15 aa, synthetic construct
  REGION 1..15: note = synthetic
  SITE 4: note = Xaa - D-Aspartic acid
  SITE 7: note = Xaa - homoarginine
CPFXCLXNWSTPIWC

SEQ ID NO: 162 - protein, 15 aa, synthetic construct
  REGION 1..15: note = synthetic
  SITE 4: note = Xaa - D-Aspartic acid
  SITE 7: note = Xaa - homoarginine
CPYXCMXNWSTPIWC

SEQ ID NO: 163 - protein, 15 aa, synthetic construct
  REGION 1..15: note = synthetic
  SITE 2: note = Xaa - Aib
  SITE 4: note = Xaa - D-Aspartic acid
  SITE 7: note = Xaa - homoarginine
CXFXCMXNWSTPIWC

SEQ ID NO: 164 - protein, 15 aa, synthetic construct
  REGION 1..15: note = synthetic
  SITE 2: note = Xaa - sarcosine
  SITE 4: note = Xaa - D-Aspartic acid
  SITE 7: note = Xaa - homoarginine
CXFXCMXNWSTPIWC

SEQ ID NO: 165 - protein, 15 aa, synthetic construct
  REGION 1..15: note = synthetic
  SITE 4: note = Xaa - D-arginine
  SITE 7: note = Xaa - homoarginine
CPFXCMXNWSTPIWC

SEQ ID NO: 166 - protein, 15 aa, synthetic construct
  REGION 1..15: note = synthetic
  SITE 4: note = Xaa - D-Aspartic acid
  SITE 7: note = Xaa - homoarginine
CPFXCMXNWSTPKWC

SEQ ID NO: 167 - protein, 15 aa, synthetic construct
  REGION 1..15: note = synthetic
  SITE 3: note = Xaa - 1-naphthyl alanine
  SITE 4: note = Xaa - D-Aspartic acid
  SITE 7: note = Xaa - homoarginine
  SITE 13: note = Xaa - hydroxyproline
CPXXCMXNWSTPXWC

SEQ ID NO: 168 - protein, 15 aa, synthetic construct
  REGION 1..15: note = synthetic
  SITE 3: note = Xaa - 1-naphthyl alanine
  SITE 4: note = Xaa - D-Aspartic acid
  SITE 7: note = Xaa - homoarginine
  SITE 13: note = Xaa - hydroxyproline
CPXXCMXHWSTPXWC

SEQ ID NO: 169 - protein, 15 aa, synthetic construct
  REGION 1..15: note = synthetic
  SITE 3: note = Xaa - 1-naphthyl alanine
  SITE 4: note = Xaa - D-Aspartic acid
  SITE 7: note = Xaa - homoarginine
  SITE 13: note = Xaa - hydroxyproline
CPXXCMXDWSTPXWC

SEQ ID NO: 170 - protein, 15 aa, synthetic construct
  REGION 1..15: note = synthetic
  SITE 3: note = Xaa - 1-naphthyl alanine
  SITE 4: note = Xaa - D-Aspartic acid
  SITE 7: note = Xaa - homoarginine
CPXXCMXDWSTPIWC

SEQ ID NO: 171 - protein, 15 aa, synthetic construct
  REGION 1..15: note = synthetic
  SITE 3: note = Xaa - 1-naphthyl alanine
  SITE 4: note = Xaa - D-arginine
  SITE 7: note = Xaa - homoarginine
  SITE 13: note = Xaa - hydroxyproline
CPXXCMXNWSTPXWC

SEQ ID NO: 172 - protein, 15 aa, synthetic construct
  REGION 1..15: note = synthetic
  SITE 3: note = Xaa - 1-naphthyl alanine
  SITE 4: note = Xaa - D-arginine
  SITE 7: note = Xaa - homoarginine
  SITE 13: note = Xaa - hydroxyproline
CPXXCMXHWSTPXWC

SEQ ID NO: 173 - protein, 15 aa, synthetic construct
  REGION 1..15: note = synthetic
  SITE 4: note = Xaa - D-Aspartic acid
  SITE 7: note = Xaa - N-methyl-homoarginine
CPFXCMXNWSTPIWC

SEQ ID NO: 174 - protein, 15 aa, synthetic construct
  REGION 1..15: note = synthetic
  SITE 4: note = Xaa - D-Aspartic acid
  SITE 7: note = Xaa - homoarginine
  SITE 8: note = Xaa - N-methyl-asparagine
CPFXCMXXWSTPIWC

SEQ ID NO: 175 - protein, 15 aa, synthetic construct
  REGION 1..15: note = synthetic
  SITE 4: note = Xaa - D-Aspartic acid
  SITE 7: note = Xaa - homoarginine
  SITE 11: note = Xaa - N-methyl-Threnine
CPFXCMXNWSXPIWC

SEQ ID NO: 176 - protein, 15 aa, synthetic construct
  REGION 1..15: note = synthetic
  SITE 4: note = Xaa - D-Aspartic acid
  SITE 7: note = Xaa - homoarginine
  SITE 13: note = Xaa - N-methyl-Ile
CPFXCMXNWSTPXWC

SEQ ID NO: 177 - protein, 15 aa, synthetic construct
  REGION 1..15: note = synthetic
  SITE 3: note = Xaa - 1-naphthyl alanine
  SITE 4: note = Xaa - D-Aspartic acid
  SITE 7: note = Xaa - homoarginine
  SITE 8: note = Xaa - cysteic acid
  SITE 13: note = Xaa - hydroxyproline
CPXXCMXXWSTPXWC

SEQ ID NO: 178 - protein, 15 aa, synthetic construct
  REGION 1..15: note = synthetic
  SITE 3: note = Xaa - 1-naphthyl alanine
  SITE 4: note = Xaa - D-Aspartic acid
  SITE 7: note = Xaa - cysteic acid
  SITE 13: note = Xaa - hydroxyproline
CPXXCMXDWSTPXWC

SEQ ID NO: 179 - protein, 15 aa, synthetic construct
  REGION 1..15: note = synthetic
  SITE 3: note = Xaa - 1-naphthyl alanine
  SITE 4: note = Xaa - D-cysteic acid
  SITE 7: note = Xaa - homoarginine
  SITE 13: note = Xaa - hydroxyproline
CPXXCMXDWSTPXWC

SEQ ID NO: 180 - protein, 15 aa, synthetic construct
  REGION 1..15: note = synthetic
  SITE 3: note = Xaa - 1-naphthyl alanine
  SITE 4: note = Xaa - D-Aspartic acid
  SITE 7: note = Xaa - homoarginine
  SITE 13: note = Xaa - hydroxyproline
CPXXCMXDWDTPXWC

SEQ ID NO: 181 - protein, 15 aa, synthetic construct
  REGION 1..15: note = synthetic
  SITE 3: note = Xaa - 2-naphthyl alanine
  SITE 4: note = Xaa - D-Aspartic acid
  SITE 7: note = Xaa - homoarginine
  SITE 13: note = Xaa - hydroxyproline
CPXXCMXDWSTPXWC

SEQ ID NO: 182 - protein, 15 aa, synthetic construct
  REGION 1..15: note = synthetic
  SITE 3: note = Xaa - 1-naphthyl alanine
  SITE 4: note = Xaa - D-Aspartic acid
  SITE 7: note = Xaa - homoarginine
  SITE 13: note = Xaa - hydroxyproline
CPXXCMXDWTTPXWC

SEQ ID NO: 183 - protein, 15 aa, synthetic construct
  REGION 1..15: note = synthetic
  SITE 3: note = Xaa - 1-naphthyl alanine
  SITE 4: note = Xaa - D-Aspartic acid
  SITE 7: note = Xaa - homoarginine
  SITE 10: note = Xaa - homoserine
  SITE 13: note = Xaa - hydroxyproline
CPXXCMXDWXTPXWC

SEQ ID NO: 184 - protein, 15 aa, synthetic construct
  REGION 1..15: note = synthetic
  SITE 3: note = Xaa - 1-naphthyl alanine
  SITE 4: note = Xaa - D-Aspartic acid
  SITE 7: note = Xaa - homoarginine
  SITE 10: note = Xaa - D-serine
  SITE 13: note = Xaa - hydroxyproline
CPXXCMXDWXTPXWC

SEQ ID NO: 185 - protein, 15 aa, synthetic construct
  REGION 1..15: note = synthetic
  SITE 3: note = Xaa - 1-naphthyl alanine
  SITE 4: note = Xaa - D-Aspartic acid
  SITE 7: note = Xaa - homoarginine
  SITE 13: note = Xaa - hydroxyproline
CPXXCMXDWSSPXWC

SEQ ID NO: 186 - protein, 15 aa, synthetic construct
  REGION 1..15: note = synthetic
  SITE 3: note = Xaa - 1-naphthyl alanine
  SITE 4: note = Xaa - D-Aspartic acid
  SITE 7: note = Xaa - 2-amino-4-guanidinobutyric acid
  SITE 13: note = Xaa - hydroxyproline
CPXXCMXDWSTPXWC

SEQ ID NO: 187 - protein, 15 aa, synthetic construct
  REGION 1..15: note = synthetic
  SITE 3: note = Xaa - 1-naphthyl alanine
  SITE 4: note = Xaa - D-Aspartic acid
  SITE 13: note = Xaa - hydroxyproline
CPXXCMPDWSTPXWC

SEQ ID NO: 188 - protein, 15 aa, synthetic construct
  REGION 1..15: note = synthetic
  SITE 3: note = Xaa - 1-naphthyl alanine
  SITE 4: note = Xaa - D-Aspartic acid
  SITE 7: note = Xaa - hydroxyproline
  SITE 13: note = Xaa - hydroxyproline
CPXXCMXDWSTPXWC

SEQ ID NO: 189 - protein, 15 aa, synthetic construct
  REGION 1..15: note = synthetic
  SITE 3: note = Xaa - 1-naphthyl alanine
  SITE 4: note = Xaa - D-arginine
  SITE 7: note = Xaa - homoarginine
  SITE 13: note = Xaa - hydroxyproline
CPXXCMXDWSTPXWC

SEQ ID NO: 190 - protein, 15 aa, synthetic construct
  REGION 1..15: note = synthetic
  SITE 3: note = Xaa - 1-naphthyl alanine
  SITE 4: note = Xaa - D-arginine
  SITE 7: note = Xaa - homoarginine
  SITE 13: note = Xaa - hydroxyproline
CPXXCMXDWDTPXWC

SEQ ID NO: 191 - protein, 15 aa, synthetic construct
  REGION 1..15: note = synthetic
  SITE 3: note = Xaa - 2-naphthyl alanine
  SITE 4: note = Xaa - D-arginine
  SITE 7: note = Xaa - homoarginine
  SITE 13: note = Xaa - hydroxyproline
CPXXCMXDWSTPXWC

SEQ ID NO: 192 - protein, 15 aa, synthetic construct
  REGION 1..15: note = synthetic
  SITE 3: note = Xaa - 1-naphthyl alanine
  SITE 4: note = Xaa - D-arginine
  SITE 7: note = Xaa - homoarginine
  SITE 13: note = Xaa - hydroxyproline
CPXXCMXDWTTPXWC

SEQ ID NO: 193 - protein, 15 aa, synthetic construct
  REGION 1..15: note = synthetic
  SITE 3: note = Xaa - 1-naphthyl alanine
  SITE 4: note = Xaa - D-arginine
  SITE 7: note = Xaa - homoarginine
  SITE 10: note = Xaa - homoserine
  SITE 13: note = Xaa - hydroxyproline
CPXXCMXDWXTPXWC

SEQ ID NO: 194 - protein, 15 aa, synthetic construct
  REGION 1..15: note = synthetic
  SITE 3: note = Xaa - 1-naphthyl alanine
  SITE 4: note = Xaa - D-arginine
  SITE 7: note = Xaa - homoarginine
  SITE 10: note = Xaa - D-serine
  SITE 13: note = Xaa - hydroxyproline
CPXXCMXDWXTPXWC

SEQ ID NO: 195 - protein, 15 aa, synthetic construct
  REGION 1..15: note = synthetic
  SITE 3: note = Xaa - 1-naphthyl alanine
  SITE 4: note = Xaa - D-arginine
  SITE 7: note = Xaa - homoarginine
  SITE 13: note = Xaa - hydroxyproline
CPXXCMXDWSSPXWC

SEQ ID NO: 196 - protein, 15 aa, synthetic construct
  REGION 1..15: note = synthetic
  SITE 3: note = Xaa - 1-naphthyl alanine
  SITE 4: note = Xaa - D-arginine
  SITE 7: note = Xaa - 2-amino-4-guanidinobutyric acid
  SITE 13: note = Xaa - hydroxyproline
CPXXCMXDWSTPXWC

SEQ ID NO: 197 - protein, 15 aa, synthetic construct
  REGION 1..15: note = synthetic
  SITE 3: note = Xaa - 1-naphthyl alanine
  SITE 4: note = Xaa - D-arginine
  SITE 13: note = Xaa - hydroxyproline
CPXXCMPDWSTPXWC

SEQ ID NO: 198 - protein, 15 aa, synthetic construct
  REGION 1..15: note = synthetic
  SITE 3: note = Xaa - 1-naphthyl alanine
  SITE 4: note = Xaa - D-arginine
  SITE 7: note = Xaa - hydroxyproline
  SITE 13: note = Xaa - hydroxyproline
CPXXCMXDWSTPXWC

SEQ ID NO: 199 - protein, 15 aa, synthetic construct
  REGION 1..15: note = synthetic
  SITE 3: note = Xaa - 1-naphthyl alanine
  SITE 4: note = Xaa - D-Aspartic acid
  SITE 7: note = Xaa - homoarginine
CPXXCLXDWSTPIWC

SEQ ID NO: 200 - protein, 15 aa, synthetic construct
  REGION 1..15: note = synthetic
  SITE 3: note = Xaa - 1-naphthyl alanine
  SITE 4: note = Xaa - D-Aspartic acid
  SITE 7: note = Xaa - homoarginine
  SITE 13: note = Xaa - hydroxyproline
CPXXCLXDWSTPXWC

SEQ ID NO: 201 - protein, 15 aa, synthetic construct
  REGION 1..15: note = synthetic
  SITE 3: note = Xaa - 1-naphthyl alanine
  SITE 4: note = Xaa - D-arginine
  SITE 7: note = Xaa - homoarginine
  SITE 13: note = Xaa - hydroxyproline
CPXXCLXDWSTPXWC

SEQ ID NO: 202 - protein, 15 aa, synthetic construct
  REGION 1..15: note = synthetic
  SITE 3: note = Xaa - 1-naphthyl alanine
  SITE 4: note = Xaa - D-arginine
  SITE 7: note = Xaa - homoarginine
  SITE 13: note = Xaa - hydroxyproline
CPXXCLXHWSTPXWC

SEQ ID NO: 203 - protein, 15 aa, synthetic construct
  REGION 1..15: note = synthetic
  SITE 3: note = Xaa - 1-naphthyl alanine
  SITE 4: note = Xaa - D-arginine
  SITE 7: note = Xaa - homoarginine
CPXXCMXDWSTPIWC

SEQ ID NO: 204 - protein, 15 aa, synthetic construct
  REGION 1..15: note = synthetic
  SITE 3: note = Xaa - F/3-methyl-phenylalanine /4-methyl-phenylalanine /homophenylalanine/4,4-biphenylalanine /3,4-dihydroxy-phenylalanine /Y/A/1-naphthyl alanine/2-naphthyl alanine/2-pyridylalanine
  SITE 4: note = Xaa - G/A/D/K/acetyl-lysine /F/E/Q/L/S/R/cysteic acid
  SITE 6: note = Xaa - absent/M/methionine sulfone/Q/homoglutamine/L/homoleucine/Nle/K/I/t-butyl-alanine/Homoserine-methyl
  SITE 7: note = Xaa - homoarginine
  SITE 8: note = Xaa - N/N-methyl-asparagine/T/D/G/S/H/A/Thienyl-alanine/3-(1,2,4-Triazol-1-yl)-alanine/Beta-(4-thiazolyl)-alanine /K/cysteic acid
  SITE 13: note = Xaa - I/N-methyl-Isoleucine/A/3-cyclohexyl-alanine /cyclopropyl-alanine /P/hydroxyproline/D/K/cyclopentyl-glycine /tetrahydropyran-4-propanoic acid /dioxo-4-tetrahydrothiopyranylacetic acid
CPXXCXXXWSTPXWC

SEQ ID NO: 205 - protein, 15 aa, synthetic construct
  REGION 1..15: note = synthetic
  SITE 3: note = Xaa - F/1-naphthyl alanine
  SITE 4: note = Xaa - D-aspartic acid/D-arginine
  SITE 6: note = Xaa - M/L
  SITE 7: note = Xaa - homoarginine
  SITE 8: note = Xaa - N/H/D
  SITE 13: note = Xaa - I/P/hydroxyproline
CPXXCXXXWSTPXWC

SEQ ID NO: 206 - skipped

SEQ ID NO: 207 - protein, 15 aa, synthetic construct
  REGION 1..15: note = synthetic
  SITE 3: note = Xaa - 1-naphthyl alanine
  SITE 4: note = Xaa - D/cysteic acid
  SITE 7: note = Xaa - homoarginine/cysteic acid
  SITE 8: note = Xaa - D/cysteic acid
  SITE 13: note = Xaa - hydroxyproline
CPXXCMXXWSTPXWC

SEQ ID NO: 208 - protein, 15 aa, synthetic construct
  REGION 1..15: note = synthetic
  SITE 3: note = Xaa - 1-naphthyl alanine
  SITE 4: note = Xaa - D-cysteic acid
  SITE 7: note = Xaa - cysteic acid
  SITE 13: note = Xaa - hydroxyproline
CPXXCMXDWSTPXWC

SEQ ID NO: 209 - protein, 15 aa, synthetic construct
  REGION 1..15: note = synthetic
  SITE 3: note = Xaa - 1-naphthyl alanine
  SITE 4: note = Xaa - D-cysteic acid
  SITE 7: note = Xaa - homoarginine
  SITE 8: note = Xaa - cysteic acid
  SITE 13: note = Xaa - hydroxyproline
CPXXCMXXWSTPXWC

SEQ ID NO: 210 - protein, 15 aa, synthetic construct
  REGION 1..15: note = synthetic
  SITE 3: note = Xaa - 1-naphthyl alanine
  SITE 4: note = Xaa - D-Aspartic acid
  SITE 7: note = Xaa - cysteic acid
  SITE 8: note = Xaa - cysteic acid
  SITE 13: note = Xaa - hydroxyproline
CPXXCMXXWSTPXWC

SEQ ID NO: 211 - protein, 15 aa, synthetic construct
  REGION 1..15: note = synthetic
  SITE 3: note = Xaa - 1-naphthyl alanine
  SITE 4: note = Xaa - D-lysine
  SITE 7: note = Xaa - homoarginine
  SITE 13: note = Xaa - hydroxyproline
CPXXCMXDWSTPXWC

SEQ ID NO: 212 - protein, 15 aa, synthetic construct
  REGION 1..15: note = synthetic
  SITE 3: note = Xaa - 1-naphthyl alanine
  SITE 4: note = Xaa - D-Aspartic acid
  SITE 13: note = Xaa - hydroxyproline
CPXXCMKDWSTPXWC

SEQ ID NO: 213 - protein, 15 aa, synthetic construct
  REGION 1..15: note = synthetic
  SITE 3: note = Xaa - F/3-methyl-phenylalanine /4-methyl-phenylalanine /homophenylalanine/4,4-biphenylalanine /3,4-dihydroxy-phenylalanine /Y/A/1-naphthyl alanine/2-naphthyl alanine/2-pyridylalanine
  SITE 4: note = Xaa - G/A/D/K/acetyl-lysine/F/E/Q/L/S/R/cysteic acid
  SITE 6: note = Xaa - absent/M/methionine sulfone/Q/homoglutamine/L/homoleucine/Nle/K/I/t-butyl-alanine/Homoserine(Me)
  SITE 7: note = Xaa - homoarginine/K
  SITE 8: note = Xaa - N/N-methyl-asparagine/T/D/G/S/H/A/Thienyl-alanine/3-(1,2,4-Triazol-1-yl)-alanine/Beta-(4-thiazolyl)-alanine /K/cysteic acid
  SITE 13: note = Xaa - I/N-methyl-Isoleucine/A/3-cyclohexyl-alanine/cyclopropyl-alanine /P/hydroxyproline/D/K/cyclopentyl-glycine/tetrahydropyran-4-propanoic acid /dioxo-4-tetrahydrothiopyranylacetic acid
CPXXCXXXWSTPXWC

SEQ ID NO: 214 - protein, 15 aa, synthetic construct
  REGION 1..15: note = synthetic
  SITE 3: note = Xaa - F/1-naphthyl alanine
  SITE 4: note = Xaa - D-aspartic acid/D-arginine
  SITE 6: note = Xaa - M/L
  SITE 7: note = Xaa - homoarginine/K
  SITE 8: note = Xaa - N/H/D
  SITE 13: note = Xaa - I/P/hydroxyproline
CPXXCXXXWSTPXWC

SEQ ID NO: 215 - protein, 15 aa, synthetic construct
  REGION 1..15: note = synthetic
  SITE 3: note = Xaa - 1-naphthyl alanine
  SITE 4: note = Xaa - D-Aspartic acid
  SITE 7: note = Xaa - homoarginine
  SITE 9: note = Xaa - D-tryptophan
  SITE 13: note = Xaa - hydroxyproline
  SITE 14: note = Xaa - D-tryptophan
CPXXCMXDXSTPXXC

SEQ ID NO: 216 - protein, 15 aa, synthetic construct
  REGION 1..15: note = synthetic
  SITE 7: note = Xaa - homoarginine
  SITE 13: note = Xaa - hydroxyproline
CPFGCMXDWSTPXWC

SEQ ID NO: 217 - protein, 24 aa, synthetic construct
  REGION 1..18: note = synthetic
  SITE 18..23: note = Xaa - sarcosine
  SITE 24: note = K(Fl)
ACPFGCHTDWSWPIWCAXXXXXXK